European Patent Application EP 4 163 277 A1, published April 12, 2023. Title: NOVEL PYRAZOLE DERIVATIVES. Applicant: APTABIO THERAPEUTICS INC. The sequence listing filed with the application follows.

SEQUENCE LISTING (6 sequences)

SEQ ID NO: 1 - DNA, 22 bp, Artificial Sequence
  IL-1 beta forward primer
ccacagaccttccaggagaatg

SEQ ID NO: 2 - DNA, 23 bp, Artificial Sequence
  IL-1 beta reverse primer
gtgcagttcagtgatcgtacagg

SEQ ID NO: 3 - DNA, 20 bp, Artificial Sequence
  GAPDH forward primer
gtggctggctcagaaaaagg

SEQ ID NO: 4 - DNA, 20 bp, Artificial Sequence
  GAPDH reverse primer
ggtggtccaggggtcttact

SEQ ID NO: 5 - DNA, 22 bp, Artificial Sequence
  Beta actin forward primer
caccattggcaatgagcggttc

SEQ ID NO: 6 - DNA, 22 bp, Artificial Sequence
  Beta actin reverse primer
aggtctttgcggatgtccacgt